European Patent Specification EP 3 786 295 B1, published October 15, 2025. Title: A method for detection of Candida auris. Applicant: Teikyo University. The sequence listing filed with the application follows.

SEQUENCE LISTING (16 sequences)

SEQ ID NO: 1 - DNA, 42 bp, Artificial sequence
aggctactgagcttgctggtgtaaccaaaccaacaggagagg

SEQ ID NO: 2 - DNA, 42 bp, Artificial sequence
acggtttcagggttagcatggctcaacaaagtcgctggtaca

SEQ ID NO: 3 - DNA, 19 bp, Artificial sequence
gggaaaggaaccctgacct

SEQ ID NO: 4 - DNA, 20 bp, Artificial sequence
ggacacagcattcgaagtgt

SEQ ID NO: 5 - DNA, 18 bp, Artificial sequence
catctcgaaggcctcggt

SEQ ID NO: 6 - DNA, 19 bp, Artificial sequence
cacatactcgaacggagtc

SEQ ID NO: 7 - DNA, 872 bp, Candida auris
cactacagcaggatcaacggatgcttcatactctgaaatcacctttaatgctgggattggcgcccacacaaagttggctgggtggacaaactcctccacagaaacagaaccgaaacggccagcgaggaacaacgaagcagcaacgtcagccttcaaggttgagccagcatccgaagataccacaacaaccttgcgtgcagacgaaggcacagaagccacgaagtgttcttgagcaaatgggaaaggaaccctgaccttaaccaaaccaacaggagaggaaaccgaggccttggagatgacaccagcaagctcagtagcctggtgagcaccaaaagcgacaaaaacagtttcagggttagcatggcccacatactcgaacggagtcaaatttgtaccagcgactttgttgaacacttcgaatgctgtgtccactgccttttccaaagaatagtcgccgtcgggaatcgaagacaccaattgctggtataagcggcccacatcggtcacagacaagatgtcatcgaacttggagatcgctttagcaaactcaggaccgtcgaaaacgtgcaaggctggtccctgaagcaaagtagccacaaagtgagtgaagatggtgatgtactgcaactccacggcgctctgcgagtccgccggggccaccacagggatacccgtggagcgagcagttgccaaaggagtcgtatagtttgaaaccaacgagtttgtttccacatcaaagtcgatagcggaaacgttcaaggtcaatggcaattttgcagccttggccaaagtgggctgcatccatggcaaggcgttggcgcccaacacagcagtatgtggtccagtggaggacacgttgctagcggcatagc

SEQ ID NO: 8 - DNA, 1533 bp, Candida auris
agtaagagctgcggtcatcaagctcaacatcttcatcgtctatcgccgacagagacgcctccatttggttttttcttgttaaattgtccaccgacaaaggctggtggcctgaagtctccgcagagtctgccataaagtttgagcaattgtagatgttgtaggttttttttgcaagtgttatcggcgtccgaagttgaagtgtgacgggcgcgcaggaaggtcagaaagcagcaaggaaacggccaaaggtaccagatagaagaaacggtctgttggggctgattttgtagaaactgatgtttaattcacattttcttcacccgtgggggttcgttgggaaccgtcacgaggcacgtttgttgtggggcacgtgtggttgcaaaatgagataagcaaggtagtgtggtttgacagcttcatataggaaggtgcaaaaaagtgcaaagagagaagaatgtaaattgaaattgtaatattccaatgagtgaagtgctaattttggaaatctgagctttttaatgtctactcaactttgatgtttcagtggatgaagcctgtttggcgtaaagtccacaggttttcggagttttggcgagcatcgacacataacaaggcaacaatgcaaagtcacgaaaatctcgaacaatggcgagtcgtaaattgggtctctgattttcctagcgtgaattgaacagaaacagtccaagtccatgcttgcattcagtcacttgttttgagatgtggccggtgagagccactgaaagcgaaccacatacatgtatccataatgtacacaataaaggctcctagatcaaaggatcaagctcataatacaagcaacaacgccatcgtgtcagccgagctatttgagtgtcacctgaagaataatacccatacttgcgctcttaagtggtagtatctgctgagcgtctatctgatctgttgaactgctaccacgagctttggggatttttcgcagcaattatacctgggcaaatacaaagcacaatattcacaagcacagcacttgtaggcgacctcatgccactggtctgattaacaaacaataagcttttgtttgataaaactaataacggatcttgcgagggtgatgtagctatgaagaacatgcatgcaacctcagccagcatgaggtattagctcgtagaatggctacgaagagacctaaacaaaagtagaagtaagtttaaagcctttccgatggaatttaacaaactacaaagtggagcaattctttttgtcggctgttatctgcttgagtggtattcatcacgctgtctgtgctcccgaggactctccgataccacaaactataatgttaaatccacatattttacatgagccgagatgaagttatgcagactcaacacaaaggaaatcaggggtcgtatcttaagttcttcttgtttctaataatcctctccagaggactccatttgcagccacaaatacctcatcgcgaaaaagtgcagcttcatctcactccataactatgtcagctgccgtcgaaac

SEQ ID NO: 9 - DNA, 1924 bp, Candida auris
atacttcaacgaaggagattacttccaatttcgaagcaaaagattggggtcagaagagcccaagtcaccaaggtcaggttatgactcgacaaagcaagcaacagccgacgaagataaatcggagggagatgaggacgatatattaaatgagggaaacctccatttccttgactttattgagaataaaacctttggtgtcaaccccagatcaaagtcggtcttcgaccgcctggcatacgactctgttgctttcatgtcgaacgatgctgaggaagaggaaaaggagaaatctctcacgactaccttagaagttcttgttgctccagattctccgcctccaagcgattacgtgatcgatcttattcacgagatatcatcaatttgcacggacgtaaaactcatgttacgttcgctcaatgtgaaacaaatgtcgaaagcgttgaagcagactgaggaggactaccacaagcttgaaagtttggctcgtcaagaacgtgaaaccgacgaagacaacaatctgcaaatcactatgaaacagacgtcacctactaggccatcggtgacgacgctaaagacgggcagtggatctgtggcttctgttccgttcaggcgtctgcaaacactggaaatcagtgagcagattccgccaccgtcgcaattgcaaggcatgagatcgtcaacatcgctcaacaccacaacatcggctctcaaattcacgcctcttaagtctgcaacaacaggtggtaaaacattttctaagggcctgctcgaagacaacaaagatttggaccggcgcattgcacaacttgtgaaagaagatgagaagaagaagctgaaggctgccaaagaagagaagcaaagattggcgaaagaagagaagctagctgctaaacaaagcaagcagagggaaaaggaaaaacaaagagaggagttgtcgcatacgaagcacaaggctactcctcttgaaaggaaccatactgagccacaagacttcttctctacgaagctgaaccgcgaagataccgatgagtcttcgttgttttcgaagccatcgatcacttcgaaagacaagaaaggaagcattatactgcggatcggacacaaactcaaacataccgagccgctcaagcacacggagtctgttgacagtgatgtgaggagtatttccacaactaaatcgtccagtagccaaacgtcaaacactagcaagaagtcgtcacgcaaggttggattatttgggttgcgcaagaggaattgagaaacaaaaggcaagagagaaaaaaaaaaaaaaaatatatatatatatactaagttggaggagaaatcaatctgctccttgtcagtgtcttttggaatgattgcatcgtaatattcttttctggagattttttttgggttttttggaacagctgcaacaccatcaacactctgagaaacaactccccgagacgcgccagctgcggctgccgcgtaggaaagttgagccccactggacttttgagaagtctgggtgccggaggagggaccttcggcgcgatttggggaggaagcaaccttagttgctttctccaggatcattggatcgctgagcagggagtttctgttctcctgacgcgtaccgccttctacggatgcgacgctagaagatacagaaacaccttttccaggacgatcaaactcgataggtggttcaggaggtcgggaatctcgctccacggtaccgggaggtcgattcgcgccttctgcttgatgccgaacgatattattcagcatttttcaaaaaggatctaagggtgtaagcttgagcttgtaaatgtattctagaacaccgaagtatttaaaactttgctttgagtcttttattgtattattaactactgtttactattgctgtcatattgaacacctttttgaaattcgccac

SEQ ID NO: 10 - DNA, 4646 bp, Candida auris
cttcgttgcgttgagaagcgccttgtccaactttttggactgctctaaaaagctgcgaagcttcttagacttggagtaaacttgtaggaatgacacggctacaccttgaagaagggtgatggggggagtgactcctccgtgaacgtagagcatgtacatgaaagttgcgtagaggccacctttcgagccggcaacaaagatctcaaatacttgtgtgtaaatgggcttgttctcccacacacgttctgaaacatcttcgtcgtcgggatcctcgtcctcatcgctgatttcctcatcattcgatacctcgttgccacccggcgacagcaatccctgattattggggatggtgtagaacatgagctcataaacgttgagtacgagtttaccgaagtatgctattgcttccatcccgagcactccgtagtggataccaaacaagagactaccaacagaacgtgtgccctggaagacgtcgtaagccaaaaacttcgctaggaggaggtcggcgacagtaaatacctcgagaagaatcagaaccctatacgtggcgaagttgtagaagacctggcgagaggttgatatctgatgcggaatcatgttcgtgattttcatctgaaacgagtcaagacggtccgtcatgatgatatgaaacactttgaacatgatcgtgaggttgatccacactatattgagaagaagattatcgtcactaaacatgattatgagaagattaataaggtagaagggtaactcctccgaaatatgctcaatttcaatgatccgaagctctctgaagatcaatttgatccctgcaaaccccatgagaataaagcaacttaccacgaagttgaggagaattaggagtctcacgctctccgtgagctcgtacatcatggtaagataatcgacagagttcatggccagaaccacgagcgatgcagcgaaaaggccgaagctaatgccgccatacactgcaattgcaatggtgccctttcgaggcatggttatggtgttttgtctttcttttgtggggacgaaaggtgtggaagccggaagtaaacacctcaccttcgcgataatcctagatctacgctaacttgcgcatagagggtcgtgcgcgcaaaattttccccagacttccaattagtggtcgcttgagtctattaaagttgcggaattcgggacttatggaggtcattgcgtaatggtgacatttcagttcgtcttcttttgatgtctggaatcatgctctgtccgtttaattgcctcataggcagcctcagtggcagtctcatgggcagtcgcagaggtgatctggatgctggtgaagttgccgggcgcttcaattgagcaggtgatctttgtagctctgacaatgattgggaaaatattttgaggttcttctcggtgtgatttaagtcgcgagaaattccgtggtagttcttatcgatcatgtcggatacaatatgtgccttttgagttgcagctttctctatagagtccgcctggctgcgactagtattggtaatatcagccaaagcattatcaataacttgtttggtctccttctgtaatcttccaaaggctccctgcacatctttggtggcaacctctttgaaggacttgagatccgtggccactgacttggtctttgttgatatcgactgtagcgtttgggaattttgatgaatgtaggcctgatactctttgcttagagttgtcttctcttcttgcatgaattctgttgcactttccctaaccgcctcggcattggcgtccttgcttgacttcacgaacccgtcaaatgctaggtgcatttgttgcatatattgctccttaagtgcctcatacgtctctgccatacgagccttgaacttcttctcaaaggccttgtacattgcggagtcttccagaagatgtgttgagttgatgtaatccgttagttgctcattcctcttgttcactccagctacgtgcagcgagaaatcgaggttttgacaaacattatgaagggtagaaaagtccatcagattagcgagaacctgctcgaaggctgatgtctccttctctactttggaagaaacatcatttaatttgccctcgagagtcttcttaaaaaggcaaagatgcgtttgaacgacggtggggatctccttcacattcagcagcacctgagttaggtcattaagattgttaatcacctcattaacgtccctaatgatactcagaattccagttcctgtaacattagagactcgctctttttgagagctgtatttgtcttttaaatgcatgaactcttttgtagtcttgtgaagctcagcgtctttagctgcgaggtccagcctgcttttcgagttctcgctaagtgtttgctcgatctgtagtttgagttctgcaatatccttgtccctcccttgaagtttggcgtgtagccctgtaatctgagtgtctttctccttcaactcggttctaagttccgcaattttcctttcaaagtcctcgtagttctgaagactgatcctgatgctgttgtctttgccttttgtagccaataagtctctattcaatctagaaatctccgctgataactcccttatctttgtacgtttgagaacgagctcgctgtcggccgtcgattgtggtatatttttgatattcttcgccttggaagcgtaagttagcgtcagcatcgtttccattaagttcagctttgccggggaaatggtagcaatcaatgcggttttggtccgccctccaatagagccttgaagaagacgggtgagtttagactctctataaggtatatgtctaggttctttgccttcactcaatgcactgatgacctttcccaaagtcaaaagactctggttgatcaggcccgcttctttggcactagcatcggtagcgccagacttgatgatatcttccagccccgcgagatccaccaaattcatttttgacagccgcaccacctcttgccctgacgacgacattactgttttgtgaagcgttatggtgaaaatggtgtgagaacgtgatgagcgggagttgagtttagtggtacccatcttcctcttccctaggcacttttgtagcatctcaaaccccagcttcgcatccaccacgtcaagctcatacaaattctggatcattgttccccttccatctctcgaaccatcccctaggagccttagtttcggcttttttgagttcaactcaagctcatcgttgacgagatcatggagctcttccttgtacaattccacacacgacaacttgacacagatgtcgtctttggccacctgaaaaagctcttgcaacacacgaggcacaatacccgcatgctctcccactaaatcccccaacattgtatacgtctttcctgagcctgtcaggccatacgcaaggatagtgacattcatgcctgccatgaaatctcgaagtaacggacgagcaatgtttttgtaaatgagttcctgatcagcattggcaccatagacttggtctagtgtaaatactttgcctgaaccgtctgatccagagccaaaggaagtgttgggggaagcattcacgctaacgtagggttcatccgtggaacagaaatcgtcaggcaccgagaccacaatcggggactgggcggctatctccagctcagttcttcttcgcacacgggcgctgacctggattttgtcggacatatagtacagttttttttttgtagtctttctttgtggagattatggtgatgtttatgtttgtttacgatgggcggcctgtgtgcaggtcggaacggtcaaagcatgtagagtgtctagagtctttatcgatgaatggaagtagaggaggtaaaattctaatagtgagattcttttttcgatggacgtgtttttgtttacgttcctcgtacttagttatgtttcgggtttaatggtgtttagtgagaaatggctgcaaaatgcaaaatgctgcgaaaaagtatagatcagagaaagacaatactactgtctgataaaaaacaaaagttgatgataagaataccagaatttgtactcacatataggaaatcacctagagtttgatatataatctgacacagcaatgtcaaaatcgcttttaccacgtgctataaaaagtttctaaggacgtcaccttctcgatataagataagcattctgtgaacggctgttaggaaagagcatagtgaggtatttcagttgaaatacgtatgccaaaaaaaaggcaaccattaattagattccacgtggttcactacactgaaaacagatgaactgtctacaatacagtctgtcagtgcaatgcctaccagttgctggtggcatagcacctcacgaatggatatattcgctaccaggttttgtacagctcaaaccactacatagctggtttctgtcaacctcgtcgctatcaactaacaaactcttttactaaaaaagagaagctcttctttcactacacgtactgtactagccttcgctcgtgtgacgattagccagccgtacttttccccatcaccgtaaaccatctattgatgttcatatatacagattccaatgacgacgccaatggcaatgccacgagcccccaaaaacctcaatcaaagaaatcatcgtcatcttcat

SEQ ID NO: 11 - DNA, 18 bp, Artificial sequence
gctatgccgctagcaacg

SEQ ID NO: 12 - DNA, 20 bp, Artificial sequence
cactacagcaggatcaacgg

SEQ ID NO: 13 - DNA, 40 bp, Artificial sequence
gtggtatcttcggatgctggctccagcgaggaacaacgaa

SEQ ID NO: 14 - DNA, 40 bp, Artificial sequence
acaaccttgcgtgcagacgaagggttcctttcccatttgc

SEQ ID NO: 15 - DNA, 19 bp, Artificial sequence
agaaacggaaccgaaacgg

SEQ ID NO: 16 - DNA, 20 bp, Artificial sequence
cctctcctgttggtttggtt